European Patent Specification EP 4 274 570 B1, published December 24, 2025. Title: MODULATORI DELL'ASSE BMP/SMAD E LORO USI. Applicant: Università degli Studi di Torino Fondazione Centro San Raffaele. The sequence listing filed with the application follows.

SEQUENCE LISTING (12 sequences)

SEQ ID NO: 1 - DNA, 20 bp, Artificial Sequence
  synthetic
agtgaggaccggctactgtg

SEQ ID NO: 2 - DNA, 20 bp, Artificial Sequence
  synthetic
gatcaaacgcttgcgaatct

SEQ ID NO: 3 - DNA, 22 bp, Artificial Sequence
  synthetic
tgacatctacaagcaggagtgc

SEQ ID NO: 4 - DNA, 19 bp, Artificial Sequence
  synthetic
tcgtcttcgtgttccttgc

SEQ ID NO: 5 - DNA, 19 bp, Artificial Sequence
  synthetic
gagaagccagggtttgagc

SEQ ID NO: 6 - DNA, 22 bp, Artificial Sequence
  synthetic
tcatacagtgtgagtgctgctg

SEQ ID NO: 7 - DNA, 22 bp, Artificial Sequence
  synthetic
gtggactgttctcacgctcaag

SEQ ID NO: 8 - DNA, 20 bp, Artificial Sequence
  synthetic
tccgtccttcgcttcatagg

SEQ ID NO: 9 - DNA, 18 bp, Artificial Sequence
  synthetic
atgggagtgcaggtggag

SEQ ID NO: 10 - DNA, 21 bp, Artificial Sequence
  synthetic
tctttccatcttcaagcatcc

SEQ ID NO: 11 - DNA, 20 bp, Artificial Sequence
  synthetic
gtgaaggtcggtgtgaacgg

SEQ ID NO: 12 - DNA, 20 bp, Artificial Sequence
  synthetic
gtgaaggtcggtgtgaacgg